European Patent Specification EP 3 990 620 B1, published December 13, 2023. Title: IN VITRO CELL CULTURE SYSTEM UNDER AEROBIC CONDITIONS SUITABLE FOR PHYSIOLOGICAL, PATHOLOGICAL, PHARMACOLOGICAL AND TOXICOLOGICAL INVESTIGATIONS. Applicant: CASREVOLUTION S.R.L. The sequence listing filed with the application follows.

SEQUENCE LISTING (4 sequences)

SEQ ID NO: 1 - DNA, 20 bp, Artificial Sequence
  Human BACE1 sense primer
tgccatctcacagtcatcca

SEQ ID NO: 2 - DNA, 20 bp, Artificial Sequence
  Human BACE1 anti-sense primer
ttgccagccttttccttctc

SEQ ID NO: 3 - DNA, 20 bp, Artificial Sequence
  Human glyceraldehyde-3-phosphate dehydrogenase (GAPDH) sense primer
atcaccatcttccaggagcg

SEQ ID NO: 4 - DNA, 20 bp, Artificial Sequence
  Human glyceraldehyde-3-phosphate dehydrogenase (GAPDH) anti-sense primer
cctgcttcaccaccttcttg